European Patent Specification EP 3 694 846 B1, published May 8, 2024. Title: HIV PROTEASE INHIBITORS. Applicant: Gilead Sciences, Inc. The sequence listing filed with the application follows.

SEQUENCE LISTING (2 sequences)

SEQ ID NO: 1 - protein, 6 aa, Artificial Sequence
  synthetic polypeptide substrate
TIXFQR

SEQ ID NO: 2 - protein, 13 aa, Artificial Sequence
  synthetic polypeptide substrate
SEVNLDAEFRKRR